European Patent Application EP 4 375 370 A1, published May 29, 2024. Title: FULLY FUNCTIONAL TAGGED RAD51 PROTEIN AND USES THEREOF. Applicant: INSTITUT CURIE. Application EP. The sequence listing filed with the application follows.

SEQUENCE LISTING (13 sequences)

SEQ ID NO: 1 - protein, 400 aa, Saccharomyces cerevisiae
MSQVQEQHISESQLQYGNGSLMSTVPADLSQSVVDGNGNGSSEDIEATNGSGDGGGLQEQAEAQGEMEDEAYDEAALGSFVPIEKLQVNGITMADVKKLRESGLHTAEAVAYAPRKDLLEIKGISEAKADKLLNEAARLVPMGFVTAADFHMRRSELICLTTGSKNLDTLLGGGVETGSITELFGEFRTGKSQLCHTLAVTCQIPLDIGGGEGKCLYIDTEGTFRPVRLVSIAQRFGLDPDDALNNVAYARAYNADHQLRLLDAAAQMMSESRFSLIVVDSVMALYRTDFSGRGELSARQMHLAKFMRALQRLADQFGVAVVVTNQVVAQVDGGMAFNPDPKKPIGGNIMAHSSTTRLGFKKGKGCQRLCKVVDSPCLPEAECVFAIYEDGVGDPREEDE

SEQ ID NO: 2 - protein, 236 aa, unidentified
VSKGEETIMSVIKPDMKIKLRMEGNVNGHAFVIEGEGSGKPFEGIQTIDLEVKEGAPLPFAYDILTTAFHYGNRVFTKYPEDIPDYFKQSFPEGYSWERSMTYEDGGICIATNDITMEEDSFINKIHFKGTNFPPNGPVMQKRTVGWEVSTEKMYVRDGVLKGDVKMKLLLKGGSHYRCDFRTTYKVKQKAVKLPDYHFVDHRIEILSHDKDYNKVKLYEHAVARNSTDSMDELYK

SEQ ID NO: 3 - protein, 226 aa, unidentified
MSAIKPDMKIKLRMEGNVNGHHFVIDGDGTGKPFEGKQSMDLEVKEGGPLPFAFDILTTAFHYGNRVFAKYPDNIQDYFKQSFPKGYSWERSLTFEDGGICNARNDITMEGDTFYNKVRFYGTNFPANGPVMQKKTLKWEPSTEKMYVRDGVLTGDIEMALLLEGNAHYRCDFRTTYKAKEKGVKLPGAHFVDHCIEILSHDKDYNKVKLYEHAVAHSGLPDNARR

SEQ ID NO: 4 - protein, 238 aa, synthetic construct
MSKGEELFTGVVPILVELDGDVNGHKFSVRGEGEGDATNGKLTLKFICTTGKLPVPWPTLVTTLTYGVQCFSRYPDHMKRHDFFKSAMPEGYVQERTISFKDDGTYKTRAEVKFEGDTLVNRIELKGIDFKEDGNILGHKLEYNFNSHNVYITADKQKNGIKANFKIRHNVEDGSVQLADHYQQNTPIGDGPVLLPDNHYLSTQSVLSKDPNEKRDHMVLLEFVTAAGITHGMDELYK

SEQ ID NO: 5 - protein, 237 aa, synthetic construct
SKGEELFTGVVPILVELDGDVNGHKFSVSGEGEGDATYGKLTLKFICTTGKLPVPWPTLVTTFGYGVQCFARYPDHMKQHDFFKSAMPEGYVQERTIFFKDDGNYKTRAEVKFEGDTLVNRIELKGIDFKEDGNILGHKLEYNYNSHNVYIMADKQKNGIKVNFKIRHNIEDGSVQLADHYQQNTPIGDGPVLLPDNHYLSTQSALSKDPNEKTDHMVLLEFVTAAGITHGMDELYK

SEQ ID NO: 6 - protein, 235 aa, unidentified
VSKGEEDNMAIIKEFMRFKVHMEGSVNGHEFEIEGEGEGRPYEGTQTAKLKVTKGGPLPFAWDILSPQFMYGSKAYVKHPADIPDYLKLSFPEGFKWERVMNFEDGGVVTVTQDSSLQDGEFIYKVKLRGTNFPSDGPVMQKKTMGWEASSERMYPEDGALKGEIKQRLKLKDGGHYDAEVKTTYKAKKPVQLPGAYNVNIKLDITSHNEDYTIVEQYERAEGRHSTGGMDELYK

SEQ ID NO: 7 - protein, 231 aa, unidentified
MSELIKENMHMKLYMEGTVDNHHFKCTSEGEGKPYEGTQTMRIKVVEGGPLPFAFDILATSFLYGSKTFINHTQGIPDFFKQSFPEGFTWERVTTYEDGGVLTATQDTSLQDGCLIYNVKIRGVNFTSNGPVMQKKTLGWEAFTETLYPADGGLEGRNDMALKLVGGSHLIANAKTTYRSKKPAKNLKMPVYYVDYRLERKEANNETYVEQHEVAVARYCDLPSKLGHKLN

SEQ ID NO: 8 - protein, 297 aa, unidentified
MAEIGTGFPFDPHYVEVLGERMHYVDVGPRDGTPVLFLHGNPTSSYVWRNIIPHVAPTHRCIAPDLIGMGKSDKPDLGYFFDDHVRFMDAFIEALGLEEVVLVIHDWGSALGFHWAKRNPERVKGIAFMEFIRPIPTWDEWPEFARETFQAFRTTDVGRKLIIDQNVFIEGTLPMGVVRPLTEVEMDHYREPFLNPVDREPLWRFPNELPIAGEPANIVALVEEYMDWLHQSPVPKLLFWGTPGVLIPPAEAARLAKSLPNCKAVDIGPGLNLLQEDNPDLIGSEIARWLSTLEISG

SEQ ID NO: 9 - protein, 11 aa, synthetic construct
GGAGSAGGAGG

SEQ ID NO: 10 - protein, 11 aa, synthetic construct
GGAGGASGAGG

SEQ ID NO: 11 - protein, 16 aa, synthetic construct
GGAGSAGGAGSSRKRS

SEQ ID NO: 12 - protein, 16 aa, synthetic construct
SRKRSSGAGSAGGAGG

SEQ ID NO: 13 - protein, 670 aa, synthetic construct
MSQVQEQHISESQLQYGNGSLMSTVPADLSQSVVDGNGNGSSEDIEATNGSGDGGGAGSAGGAGNRKRNGMSKGEELFTGVVPILVELDGDVNGHKFSVRGEGEGDATNGKLTLKFICTTGKLPVPWPTLVTTLTYGVQCFSRYPDHMKRHDFFKSAMPEGYVQERTISFKDDGTYKTRAEVKFEGDTLVNRIELKGIDFKEDGNILGHKLEYNFNSHNVYITADKQKNGIKANFKIRHNVEDGSVQLADHYQQNTPIGDGPVLLPDNHYLSTQSVLSKDPNEKRDHMVLLEFVTAAGITHGMDELYKGNRKRNGAGSAGGAGGGGLQEQAEAQGEMEDEAYDEAALGSFVPIEKLQVNGITMADVKKLRESGLHTAEAVAYAPRKDLLEIKGISEAKADKLLNEAARLVPMGFVTAADFHMRRSELICLTTGSKNLDTLLGGGVETGSITELFGEFRTGKSQLCHTLAVTCQIPLDIGGGEGKCLYIDTEGTFRPVRLVSIAQRFGLDPDDALNNVAYARAYNADHQLRLLDAAAQMMSESRFSLIVVDSVMALYRTDFSGRGELSARQMHLAKFMRALQRLADQFGVAVVVTNQVVAQVDGGMAFNPDPKKPIGGNIMAHSSTTRLGFKKGKGCQRLCKVVDSPCLPEAECVFAIYEDGVGDPREEDE